European Patent Application EP 4 227 316 A1, published August 16, 2023. Title: T CELL RECEPTORS, IMMUNE CELL COMPRISING T CELL RECEPTORS AND METHOD USING THE SAME. Applicant: Industy-Academic Cooperation foundation Yonsei University. The sequence listing filed with the application follows.

SEQUENCE LISTING (58 sequences)

SEQ ID NO: 1 - protein, 15 aa, Artificial Sequence
  amino acid sequence of the CDR3 regions in TCR alpha
CAFIGHGGSQGNLIF

SEQ ID NO: 2 - protein, 11 aa, Artificial Sequence
  amino acid sequence of the CDR3 regions in TCR alpha
CAATGTYKYIF

SEQ ID NO: 3 - protein, 12 aa, Artificial Sequence
  amino acid sequence of the CDR3 regions in TCR alpha
CAYGGGSEKLVF

SEQ ID NO: 4 - protein, 10 aa, Artificial Sequence
  amino acid sequence of the CDR3 regions in TCR alpha
CALINARLMF

SEQ ID NO: 5 - protein, 13 aa, Artificial Sequence
  amino acid sequence of the CDR3 regions in TCR alpha
CAVNGGSQGNLIF

SEQ ID NO: 6 - protein, 16 aa, Artificial Sequence
  amino acid sequence of the CDR3 regions in TCR alpha
CAMREGYGGATNKLIF

SEQ ID NO: 7 - protein, 16 aa, Artificial Sequence
  amino acid sequence of the CDR3 regions in TCR alpha
CAYNNGDGGSQGNLIF

SEQ ID NO: 8 - protein, 13 aa, Artificial Sequence
  amino acid sequence of the CDR3 regions in TCR alpha
CATDGGSARQLTF

SEQ ID NO: 9 - protein, 12 aa, Artificial Sequence
  amino acid sequence of the CDR3 regions in TCR alpha
CATLYNTDKLIF

SEQ ID NO: 10 - protein, 19 aa, Artificial Sequence
  amino acid sequence of the CDR3 regions in TCR alpha
CAMRGPWRGSSGSARQLTF

SEQ ID NO: 11 - protein, 17 aa, Artificial Sequence
  amino acid sequence of the CDR3 regions in TCR alpha
CALSVRGFKTSYDKVIF

SEQ ID NO: 12 - protein, 14 aa, Artificial Sequence
  amino acid sequence of the CDR3 regions in TCR alpha
CAVNMMDSSYKLIF

SEQ ID NO: 13 - protein, 14 aa, Artificial Sequence
  amino acid sequence of the CDR3 regions in TCR beta
CASSMQGAMSEQFF

SEQ ID NO: 14 - protein, 18 aa, Artificial Sequence
  amino acid sequence of the CDR3 regions in TCR beta
CASSPEFARALDNQPQHF

SEQ ID NO: 15 - protein, 14 aa, Artificial Sequence
  amino acid sequence of the CDR3 regions in TCR beta
CASSSATGTQGYTF

SEQ ID NO: 16 - protein, 13 aa, Artificial Sequence
  amino acid sequence of the CDR3 regions in TCR beta
CASSFTNTGELFF

SEQ ID NO: 17 - protein, 14 aa, Artificial Sequence
  amino acid sequence of the CDR3 regions in TCR beta
CASSMWQGNGEQYF

SEQ ID NO: 18 - protein, 17 aa, Artificial Sequence
  amino acid sequence of the CDR3 regions in TCR beta
CASSVGPGTTSYNEQFF

SEQ ID NO: 19 - protein, 14 aa, Artificial Sequence
  amino acid sequence of the CDR3 regions in TCR beta
CATSRDRSTDTQYF

SEQ ID NO: 20 - protein, 12 aa, Artificial Sequence
  amino acid sequence of the CDR3 regions in TCR beta
CASSLGLSGYTF

SEQ ID NO: 21 - protein, 13 aa, Artificial Sequence
  amino acid sequence of the CDR3 regions in TCR beta
CASSQSMNTEAFF

SEQ ID NO: 22 - protein, 13 aa, Artificial Sequence
  amino acid sequence of the CDR3 regions in TCR beta
CASRTGLSYEQYF

SEQ ID NO: 23 - protein, 14 aa, Artificial Sequence
  amino acid sequence of the CDR3 regions in TCR beta
CASSFGSAYNEQFF

SEQ ID NO: 24 - protein, 16 aa, Artificial Sequence
  amino acid sequence of the CDR3 regions in TCR beta
CASSFPTARSNTEAFF

SEQ ID NO: 25 - DNA, 45 bp, Artificial Sequence
  Nucleotide sequence of the CDR3 regions in TCR alpha
tgtgcctttataggccatggaggaagccaaggaaatctcatcttt

SEQ ID NO: 26 - DNA, 33 bp, Artificial Sequence
  Nucleotide sequence of the CDR3 regions in TCR alpha
tgtgcagcaacaggaacctacaaatacatcttt

SEQ ID NO: 27 - DNA, 36 bp, Artificial Sequence
  Nucleotide sequence of the CDR3 regions in TCR alpha
tgtgcttatggcggcggatctgaaaagctggtcttt

SEQ ID NO: 28 - DNA, 30 bp, Artificial Sequence
  Nucleotide sequence of the CDR3 regions in TCR alpha
tgtgctctgattaatgccagactcatgttt

SEQ ID NO: 29 - DNA, 39 bp, Artificial Sequence
  Nucleotide sequence of the CDR3 regions in TCR alpha
tgtgccgtgaacggaggaagccaaggaaatctcatcttt

SEQ ID NO: 30 - DNA, 48 bp, Artificial Sequence
  Nucleotide sequence of the CDR3 regions in TCR alpha
tgtgcaatgagagagggatatggtggtgctacaaacaagctcatcttt

SEQ ID NO: 31 - DNA, 48 bp, Artificial Sequence
  Nucleotide sequence of the CDR3 regions in TCR alpha
tgtgcttataataacggggatggaggaagccaaggaaatctcatcttt

SEQ ID NO: 32 - DNA, 39 bp, Artificial Sequence
  Nucleotide sequence of the CDR3 regions in TCR alpha
tgtgctacggacgggggttctgcaaggcaactgaccttt

SEQ ID NO: 33 - DNA, 36 bp, Artificial Sequence
  Nucleotide sequence of the CDR3 regions in TCR alpha
tgtgctacgttatataacaccgacaagctcatcttt

SEQ ID NO: 34 - DNA, 57 bp, Artificial Sequence
  Nucleotide sequence of the CDR3 regions in TCR alpha
tgtgcaatgagagggccctggagagggtcttctggttctgcaaggcaactgaccttt

SEQ ID NO: 35 - DNA, 51 bp, Artificial Sequence
  Nucleotide sequence of the CDR3 regions in TCR alpha
tgtgctctaagtgtcaggggattcaaaacctcctacgacaaggtgatattt

SEQ ID NO: 36 - DNA, 42 bp, Artificial Sequence
  Nucleotide sequence of the CDR3 regions in TCR alpha
tgtgccgtgaacatgatggatagcagctataaattgatcttc

SEQ ID NO: 37 - DNA, 42 bp, Artificial Sequence
  Nucleotide sequence of the CDR3 regions in TCR beta
tgtgccagtagtatgcagggggctatgagtgagcagttcttc

SEQ ID NO: 38 - DNA, 54 bp, Artificial Sequence
  Nucleotide sequence of the CDR3 regions in TCR beta
tgtgccagctcaccggagtttgcgagggcgctggacaatcagccccagcatttt

SEQ ID NO: 39 - DNA, 42 bp, Artificial Sequence
  Nucleotide sequence of the CDR3 regions in TCR beta
tgtgccagcagctcggccacagggacgcagggctacaccttc

SEQ ID NO: 40 - DNA, 39 bp, Artificial Sequence
  Nucleotide sequence of the CDR3 regions in TCR beta
tgtgccagcagtttcaccaacaccggggagctgtttttt

SEQ ID NO: 41 - DNA, 42 bp, Artificial Sequence
  Nucleotide sequence of the CDR3 regions in TCR beta
tgtgccagtagtatgtggcaggggaacggcgagcagtacttc

SEQ ID NO: 42 - DNA, 51 bp, Artificial Sequence
  Nucleotide sequence of the CDR3 regions in TCR beta
tgtgccagcagcgtaggcccagggacaacctcctacaatgagcagttcttc

SEQ ID NO: 43 - DNA, 42 bp, Artificial Sequence
  Nucleotide sequence of the CDR3 regions in TCR beta
tgtgccaccagcagagaccgtagcacagatacgcagtatttt

SEQ ID NO: 44 - DNA, 36 bp, Artificial Sequence
  Nucleotide sequence of the CDR3 regions in TCR beta
tgtgccagcagcttgggattaagtggctacaccttc

SEQ ID NO: 45 - DNA, 39 bp, Artificial Sequence
  Nucleotide sequence of the CDR3 regions in TCR beta
tgtgccagcagccagtcaatgaacactgaagctttcttt

SEQ ID NO: 46 - DNA, 39 bp, Artificial Sequence
  Nucleotide sequence of the CDR3 regions in TCR beta
tgtgccagcagaacgggactctcatacgagcagtacttc

SEQ ID NO: 47 - DNA, 42 bp, Artificial Sequence
  Nucleotide sequence of the CDR3 regions in TCR beta
tgtgccagcagttttgggtcagcctacaatgagcagttcttc

SEQ ID NO: 48 - DNA, 48 bp, Artificial Sequence
  Nucleotide sequence of the CDR3 regions in TCR beta
tgtgccagcagtttcccgacagctcgatcgaacactgaagctttcttt

SEQ ID NO: 49 - protein, 9 aa, homo sapiens
HVKITDFGR

SEQ ID NO: 50 - DNA, 12458 bp, Artificial Sequence
  Lentiviral vector
acgcgtgtagtcttatgcaatactcttgtagtcttgcaacatggtaacgatgagttagcaacatgccttacaaggagagaaaaagcaccgtgcatgccgattggtggaagtaaggtggtacgatcgtgccttattaggaaggcaacagacgggtctgacatggattggacgaaccactgaattgccgcattgcagagatattgtatttaagtgcctagctcgatacaataaacgggtctctctggttagaccagatctgagcctgggagctctctggctaactagggaacccactgcttaagcctcaataaagcttgccttgagtgcttcaagtagtgtgtgcccgtctgttgtgtgactctggtaactagagatccctcagacccttttagtcagtgtggaaaatctctagcagtggcgcccgaacagggacctgaaagcgaaagggaaaccagagctctctcgacgcaggactcggcttgctgaagcgcgcacggcaagaggcgaggggcggcgactggtgagtacgccaaaaattttgactagcggaggctagaaggagagagatgggtgcgagagcgtcagtattaagcgggggagaattagatcgcgatgggaaaaaattcggttaaggccagggggaaagaaaaaatataaattaaaacatatagtatgggcaagcagggagctagaacgattcgcagttaatcctggcctgttagaaacatcagaaggctgtagacaaatactgggacagctacaaccatcccttcagacaggatcagaagaacttagatcattatataatacagtagcaaccctctattgtgtgcatcaaaggatagagataaaagacaccaaggaagctttagacaagatagaggaagagcaaaacaaaagtaagaccaccgcacagcaagcggccactgatcttcagacctggaggaggagatatgagggacaattggagaagtgaattatataaatataaagtagtaaaaattgaaccattaggagtagcacccaccaaggcaaagagaagagtggtgcagagagaaaaaagagcagtgggaataggagctttgttccttgggttcttgggagcagcaggaagcactatgggcgcagcgtcaatgacgctgacggtacaggccagacaattattgtctggtatagtgcagcagcagaacaatttgctgagggctattgaggcgcaacagcatctgttgcaactcacagtctggggcatcaagcagctccaggcaagaatcctggctgtggaaagatacctaaaggatcaacagctcctggggatttggggttgctctggaaaactcatttgcaccactgctgtgccttggaatgctagttggagtaataaatctctggaacagatttggaatcacacgacctggatggagtgggacagagaaattaacaattacacaagcttaatacactccttaattgaagaatcgcaaaaccagcaagaaaagaatgaacaagaattattggaattagataaatgggcaagtttgtggaattggtttaacataacaaattggctgtggtatataaaattattcataatgatagtaggaggcttggtaggtttaagaatagtttttgctgtactttctatagtgaatagagttaggcagggatattcaccattatcgtttcagacccacctcccaaccccgaggggacccgacaggcccgaaggaatagaagaagaaggtggagagagagacagagacagatccattcgattagtgaacggatctcgacggtatcggttaacttttaaaagaaaaggggggattggggggtacagtgcaggggaaagaatagtagacataatagcaacagacatacaaactaaagaattacaaaaacaaattacaaaattcaaaattttatcgatactagtattatgcccagtacatgaccttatgggactttcctacttggcagtacatctacgtattagtcatcgctattaccatggtgatgcggttttggcagtacatcaatgggcgtggatagcggtttgactcacggggatttccaagtctccaccccattgacgtcaatgggagtttgttttggcaccaaaatcaacgggactttccaaaatgtcgtaacaactccgccccattgacgcaaatgggcggtaggcgtgtacggtgggaggtttatataagcagagctcgtttagtgaaccgtcagatcgcctggagacgccatccacgctgttttgacctccatagaagattctagagccaccatggaacatagcacgtttctctctggcctggtactggctacccttctctcgcaagtgagccccttcaagatacctatagaggaacttgaggacagagtgtttgtgaattgcaataccagcatcacatgggtagagggaacggtgggaacactgctctcagacattacaagactggacctgggaaaacgcatcctggacccacgaggaatatataggtgtaatgggacagatatatacaaggacaaagaatctaccgtgcaagttcattatcgaatgtgccagagctgtgtggagctggatccagccaccgtggctggcatcattgtcactgatgtcattgccactctgctccttgctttgggagtcttctgctttgctggacatgagactggaaggctgtctggggctgccgacacacaagctctgttgaggaatgaccaggtctatcagcccctccgagatcgagatgatgctcagtacagccaccttggaggaaactgggctcggaacaaggggtccggcggaagcggagagggcaggggatctctccttacttgtggcgacgtggaggagaaccccggccccatggaacaggggaagggcctggctgtcctcatcctggctatcattcttcttcaaggtactttggcccagtcaatcaaaggaaaccacttggttaaggtgtatgactatcaagaagatggttcggtacttctgacttgtgatgcagaagccaaaaatatcacatggtttaaagatgggaagatgatcggcttcctaactgaagataaaaaaaaatggaatctgggaagtaatgccaaggaccctcgagggatgtatcagtgtaaaggatcacagaacaagtcaaaaccactccaagtgtattacagaatgtgtcagaactgcattgaactaaatgcagccaccatatctggctttctctttgctgaaatcgtcagcattttcgtccttgctgttggggtctacttcattgctggacaggatggagttcgccagtcgagagcttcagacaagcagactctgttgcccaatgaccagctctaccagcccctcaaggatcgagaagatgaccagtacagccaccttcaaggaaaccagttgaggaggaatgggtccggcggaagcggagccaccaacttcagcctgctgaagcaggccggcgacgtggaggagaaccccggccccatgcagtcgggcactcactggagagttctgggcctctgcctcttatcagttggcgtttgggggcaagatggtaatgaagaaatgggtggtattacacagacaccatataaagtctccatctctggaaccacagtaatattgacatgccctcagtatcctggatctgaaatactatggcaacacaatgataaaaacataggcggtgatgaggatgataaaaacataggcagtgatgaggatcacctgtcactgaaggaattttcagaattggagcaaagtggttattatgtctgctaccccagaggaagcaaaccagaagatgcgaacttttatctctacctgagggcaagagtgtgtgagaactgcatggagatggatgtgatgtcggtggccacaattgtcatagtggacatctgcatcactgggggcttgctgctgctggtttactactggagcaagaatagaaaggccaaggccaagcctgtgacacgaggagcgggtgctggcggcaggcaaaggggacaaaacaaggagaggccaccacctgttcccaacccagactatgagcccatccggaaaggccagcgggacctgtattctggcctgaatcagagacgcatcggatccgggtccggcggaagcggacagtgtactaattatgctctcttgaaattggctggagatgttgagagcaaccctggacctatgaagtggaaggcgcttttcaccgcggccatcctgcaggcacagttgccgattacagaggcacagagctttggcctgctggatcccaaactctgctacctgctggatggaatcctcttcatctatggtgtcattctcactgccttgttcctgaggagtaagaggagcaggggaggtcacagtgactacatgaacatgactccccgccgccccgggcccacccgcaagcattaccagccctatgccccaccacgcgacttcgcagcctatcgctccaaacggggcagaaagaaactcctgtatatattcaaacaaccatttatgagaccagtacaaactactcaagaggaagatggctgtagctgccgatttccagaagaagaagaaggaggatgtgaactgcgggtgaagttcagcagaagcgccgacgcccctgcctaccagcagggccagaatcagctgtacaacgagctgaacctgggcagaagggaagagtacgacgtcctggataagcggagaggccgggaccctgagatgggcggcaagcctcggcggaagaacccccaggaaggcctgtataacgaactgcagaaagacaagatggccgaggcctacagcgagatcggcatgaagggcgagcggaggcggggcaagggccacgacggcctgtatcagggcctgtccaccgccaccaaggatacctacgacgccctgcacatgcaggccctgccccctcgctaacccctctccctcccccccccctaacgttactggccgaagccgcttggaataaggccggtgtgcgtttgtctatatgttattttccaccatattgccgtcttttggcaatgtgagggcccggaaacctggccctgtcttcttgacgagcattcctaggggtctttcccctctcgccaaaggaatgcaaggtctgttgaatgtcgtgaaggaagcagttcctctggaagcttcttgaagacaaacaacgtctgtagcgaccctttgcaggcagcggaaccccccacctggcgacaggtgcctctgcggccaaaagccacgtgtataagatacacctgcaaaggcggcacaaccccagtgccacgttgtgagttggatagttgtggaaagagtcaaatggctctcctcaagcgtattcaacaaggggctgaaggatgcccagaaggtaccccattgtatgggatctgatctggggcctcggtacacatgctttacatgtgtttagtcgaggttaaaaaaacgtctaggccccccgaaccacggggacgtggttttcctttgaaaaacacgatgataatatggccacaaccatggagaccctcttgggcctgcttatcctttggctgcagctgcaatgggtgagcagcaaacaggaggtgacgcagattcctgcagctctgagtgtcccagaaggagaaaacttggttctcaactgcagtttcactgatagcgctatttacaacctccagtggtttaggcaggaccctgggaaaggtctcacatctctgttgcttattcagtcaagtcagagagagcaaacaagtggaagacttaatgcctcgctggataaatcatcaggacgtagtactttatacattgcagcttctcagcctggtgactcagccacctacctctgtgcttttataggccatggaggaagccaaggaaatctcatctttggaagaggaaccagccttattgttcatccgtatatccagaaccctgaccctgccgtgtaccagctgagagactctaaatccagtgacaagtctgtctgcctattcaccgattttgattctcaaacaaatgtgtcacaaagtaaggattctgatgtgtatatcacagacaaaactgtgctagacatgaggtctatggacttcaagagcaacagtgctgtggcctggagcaacaaatctgactttgcatgtgcaaacgccttcaacaacagcattattccagaagacaccttcttccccagcccagaaagttcctgtgatgtcaagctggtcgagaaaagctttgaaacagatacgaacctaaactttcaaaacctgtcagtgattgggttccgaatcctcctcctgaaagtggccgggtttaatctgctcatgacgctgcggctgtggtccagcggaagcggagtgaaacagactttgaattttgaccttctcaagttggcgggagacgtggagtccaacccagggcccatgagcatcggcctcctgtgctgtgcagccttgtctctcctgtgggcaggtccagtgaatgctggtgtcactcagaccccaaaattccaggtcctgaagacaggacagagcatgacactgcagtgtgcccaggatatgaaccatgaatacatgtcctggtatcgacaagacccaggcatggggctgaggctgattcattactcagttggtgctggtatcactgaccaaggagaagtccccaatggctacaatgtctccagatcaaccacagaggatttcccgctcaggctgctgtcggctgctccctcccagacatctgtgtacttctgtgccagcagtatgcagggggctatgagtgagcagttctttggcccaggcacccggctgacagtgctcgaggacctgaaaaacgtgttcccacccgaggtcgctgtgtttgagccatcagaagcagagatctcccacacccaaaaggccacactggtatgcctggccacaggcttctaccccgaccacgtggagctgagctggtgggtgaatgggaaggaggtgcacagtggggtcagcacagacccgcagcccctcaaggagcagcccgccctcaatgactccagatactgcctgagcagccgcctgagggtctcggccaccttctggcagaacccccgcaaccacttccgctgtcaagtccagttctacgggctctcggagaatgacgagtggacccaggatagggccaaacccgtcacccagatcgtcagcgccgaggcctggggtagagcagactgtggcttcacctccgagtcttaccagcaaggggtcctgtctgccaccatcctctatgagatcttgctagggaaggccaccttgtatgccgtgctggtcagtgccctcgtgctgatggccatggtcaagagaaaggattccagaggctaggaattcgaatttaaatcggatccgcggccgcgaaggatctgcgatcgctccggtgcccgtcagtgggcagagcgcacatcgcccacagtccccgagaagttggggggaggggtcggcaattgaacgggtgcctagagaaggtggcgcggggtaaactgggaaagtgatgtcgtgtactggctccgcctttttcccgagggtgggggagaaccgtatataagtgcagtagtcgccgtgaacgttctttttcgcaacgggtttgccgccagaacacagctgaagcttcgaggggctcgcatctctccttcacgcgcccgccgccctacctgaggccgccatccacgccggttgagtcgcgttctgccgcctcccgcctgtggtgcctcctgaactgcgtccgccgtctaggtaagtttaaagctcaggtcgagaccgggcctttgtccggcgctcccttggagcctacctagactcagccggctctccacgctttgcctgaccctgcttgctcaactctacgtctttgtttcgttttctgttctgcgccgttacagatccaagctgtgaccggcgcctacgctagatgaccgagtacaagcccacggtgcgcctcgccacccgcgacgacgtccccagggccgtacgcaccctcgccgccgcgttcgccgactaccccgccacgcgccacaccgtcgatccggaccgccacatcgagcgggtcaccgagctgcaagaactcttcctcacgcgcgtcgggctcgacatcggcaaggtgtgggtcgcggacgacggcgccgcggtggcggtctggaccacgccggagagcgtcgaagcgggggcggtgttcgccgagatcggcccgcgcatggccgagttgagcggttcccggctggccgcgcagcaacagatggaaggcctcctggcgccgcaccggcccaaggagcccgcgtggttcctggccaccgtcggcgtctcgcccgaccaccagggcaagggtctgggcagcgccgtcgtgctccccggagtggaggcggccgagcgcgccggggtgcccgccttcctggagacctccgcgccccgcaacctccccttctacgagcggctcggcttcaccgtcaccgccgacgtcgaggtgcccgaaggaccgcgcacctggtgcatgacccgcaagcccggtgcctgagtcgacaatcaacctctggattacaaaatttgtgaaagattgactggtattcttaactatgttgctccttttacgctatgtggatacgctgctttaatgcctttgtatcatgctattgcttcccgtatggctttcattttctcctccttgtataaatcctggttgctgtctctttatgaggagttgtggcccgttgtcaggcaacgtggcgtggtgtgcactgtgtttgctgacgcaacccccactggttggggcattgccaccacctgtcagctcctttccgggactttcgctttccccctccctattgccacggcggaactcatcgccgcctgccttgcccgctgctggacaggggctcggctgttgggcactgacaattccgtggtggttgtcggggaaatcatcgtcctttccttggctgctcgcctgtgttgccacctggattctgcgcgggacgtccttctgctacgtcccttcggccctcaatccagcggaccttccttcccgcggcctgctgccggctctgcggcctcttccgcgtcttcgccttcgccctcagacgagtcggatctccctttgggccgcctccccgcctggtacctttaagaccaatgacttacaaggcagctgtagatcttagccactttttaaaagaaaaggggggactggaagggctaattcactcccaacgaagataagatctgctttttgcttgtactgggtctctctggttagaccaaatcggagcctgggagctctctggctaactagggaacccactgcttaagcctcaataaagcttgccttgagtgcttcaagtagtgtgtgcccgtctgttgtgtgactctggtaactagagatccctcagacccttttagtcagtgtggaaaatctctagcagtagtagttcatgtcatcttattattcagtatttataacttgcaaagaaatgaatatcagagagtgagaggaacttgtttattgcagcttataatggttacaaataaagcaatagcatcacaaatttcacaaataaagcatttttttcactgcattctagttgtggtttgtccaaactcatcaatgtatcttatcatgtctggctctagctatcccgcccctaactccgcccagttccgcccattctccgccccatggctgactaattttttttatttatgcagaggccgaggccgcctcggcctctgagctattccagaagtagtgaggaggcttttttggaggcctagacttttgcagagacggcccaaattcgtaatcatggtcatagctgtttcctgtgtgaaattgttatccgctcacaattccacacaacatacgagccggaagcataaagtgtaaagcctggggtgcctaatgagtgagctaactcacattaattgcgttgcgctcactgcccgctttccagtcgggaaacctgtcgtgccagctgcattaatgaatcggccaacgcgcggggagaggcggtttgcgtattgggcgctcttccgcttcctcgctcactgactcgctgcgctcggtcgttcggctgcggcgagcggtatcagctcactcaaaggcggtaatacggttatccacagaatcaggggataacgcaggaaagaacatgtgagcaaaaggccagcaaaaggccaggaaccgtaaaaaggccgcgttgctggcgtttttccataggctccgcccccctgacgagcatcacaaaaatcgacgctcaagtcagaggtggcgaaacccgacaggactataaagataccaggcgtttccccctggaagctccctcgtgcgctctcctgttccgaccctgccgcttaccggatacctgtccgcctttctcccttcgggaagcgtggcgctttctcatagctcacgctgtaggtatctcagttcggtgtaggtcgttcgctccaagctgggctgtgtgcacgaaccccccgttcagcccgaccgctgcgccttatccggtaactatcgtcttgagtccaacccggtaagacacgacttatcgccactggcagcagccactggtaacaggattagcagagcgaggtatgtaggcggtgctacagagttcttgaagtggtggcctaactacggctacactagaaggacagtatttggtatctgcgctctgctgaagccagttaccttcggaaaaagagttggtagctcttgatccggcaaacaaaccaccgctggtagcggtggtttttttgtttgcaagcagcagattacgcgcagaaaaaaaggatctcaagaagatcctttgatcttttctacggggtctgacgctcagtggaacgaaaactcacgttaagggattttggtcatgagattatcaaaaaggatcttcacctagatccttttaaattaaaaatgaagttttaaatcaatctaaagtatatatgagtaaacttggtctgacagttaccaatgcttaatcagtgaggcacctatctcagcgatctgtctatttcgttcatccatagttgcctgactccccgtcgtgtagataactacgatacgggagggcttaccatctggccccagtgctgcaatgataccgcgagacccacgctcaccggctccagatttatcagcaataaaccagccagccggaagggccgagcgcagaagtggtcctgcaactttatccgcctccatccagtctattaattgttgccgggaagctagagtaagtagttcgccagttaatagtttgcgcaacgttgttgccattgctacaggcatcgtggtgtcacgctcgtcgtttggtatggcttcattcagctccggttcccaacgatcaaggcgagttacatgatcccccatgttgtgcaaaaaagcggttagctccttcggtcctccgatcgttgtcagaagtaagttggccgcagtgttatcactcatggttatggcagcactgcataattctcttactgtcatgccatccgtaagatgcttttctgtgactggtgagtactcaaccaagtcattctgagaatagtgtatgcggcgaccgagttgctcttgcccggcgtcaatacgggataataccgcgccacatagcagaactttaaaagtgctcatcattggaaaacgttcttcggggcgaaaactctcaaggatcttaccgctgttgagatccagttcgatgtaacccactcgtgcacccaactgatcttcagcatcttttactttcaccagcgtttctgggtgagcaaaaacaggaaggcaaaatgccgcaaaaaagggaataagggcgacacggaaatgttgaatactcatactcttcctttttcaatattattgaagcatttatcagggttattgtctcatgagcggatacatatttgaatgtatttagaaaaataaacaaataggggttccgcgcacatttccccgaaaagtgccacctgacgtctaagaaaccattattatcatgacattaacctataaaaataggcgtatcacgaggccctttcgtctcgcgcgtttcggtgatgacggtgaaaacctctgacacatgcagctcccggagacggtcacagcttgtctgtaagcggatgccgggagcagacaagcccgtcagggcgcgtcagcgggtgttggcgggtgtcggggctggcttaactatgcggcatcagagcagattgtactgagagtgcaccatatgcggtgtgaaataccgcacagatgcgtaaggagaaaataccgcatcaggcgccattcgccattcaggctgcgcaactgttgggaagggcgatcggtgcgggcctcttcgctattacgccagctggcgaaagggggatgtgctgcaaggcgattaagttgggtaacgccagggttttcccagtcacgacgttgtaaaacgacggccagtgccaagctg

SEQ ID NO: 51 - DNA, 810 bp, Artificial Sequence
  T cell receptor alpha TRAV23 DV6
atggagaccctcttgggcctgcttatcctttggctgcagctgcaatgggtgagcagcaaacaggaggtgacgcagattcctgcagctctgagtgtcccagaaggagaaaacttggttctcaactgcagtttcactgatagcgctatttacaacctccagtggtttaggcaggaccctgggaaaggtctcacatctctgttgcttattcagtcaagtcagagagagcaaacaagtggaagacttaatgcctcgctggataaatcatcaggacgtagtactttatacattgcagcttctcagcctggtgactcagccacctacctctgtgcagcaacaggaacctacaaatacatctttggaagaggaaccagccttattgttcatccgtatatccagaaccctgaccctgccgtgtaccagctgagagactctaaatccagtgacaagtctgtctgcctattcaccgattttgattctcaaacaaatgtgtcacaaagtaaggattctgatgtgtatatcacagacaaaactgtgctagacatgaggtctatggacttcaagagcaacagtgctgtggcctggagcaacaaatctgactttgcatgtgcaaacgccttcaacaacagcattattccagaagacaccttcttccccagcccagaaagttcctgtgatgtcaagctggtcgagaaaagctttgaaacagatacgaacctaaactttcaaaacctgtcagtgattgggttccgaatcctcctcctgaaagtggccgggtttaatctgctcatgacgctgcggctgtggtccagc

SEQ ID NO: 52 - DNA, 948 bp, Artificial Sequence
  T cell receptor beta TRBV18
atgagcatcggcctcctgtgctgtgcagccttgtctctcctgtgggcaggtccagtgaatgctggtgtcactcagaccccaaaattccaggtcctgaagacaggacagagcatgacactgcagtgtgcccaggatatgaaccatgaatacatgtcctggtatcgacaagacccaggcatggggctgaggctgattcattactcagttggtgctggtatcactgaccaaggagaagtccccaatggctacaatgtctccagatcaaccacagaggatttcccgctcaggctgctgtcggctgctccctcccagacatctgtgtacttctgtgccagctcaccggagtttgcgagggcgctggacaatcagccccagcattttggcccaggcacccggctgacagtgctcgaggacctgaaaaacgtgttcccacccgaggtcgctgtgtttgagccatcagaagcagagatctcccacacccaaaaggccacactggtatgcctggccacaggcttctaccccgaccacgtggagctgagctggtgggtgaatgggaaggaggtgcacagtggggtcagcacagacccgcagcccctcaaggagcagcccgccctcaatgactccagatactgcctgagcagccgcctgagggtctcggccaccttctggcagaacccccgcaaccacttccgctgtcaagtccagttctacgggctctcggagaatgacgagtggacccaggatagggccaaacccgtcacccagatcgtcagcgccgaggcctggggtagagcagactgtggcttcacctccgagtcttaccagcaaggggtcctgtctgccaccatcctctatgagatcttgctagggaaggccaccttgtatgccgtgctggtcagtgccctcgtgctgatggccatggtcaagagaaaggattccagaggctag

SEQ ID NO: 53 - DNA, 822 bp, Artificial Sequence
  T cell receptor alpha TRAV24
atggagaccctcttgggcctgcttatcctttggctgcagctgcaatgggtgagcagcaaacaggaggtgacgcagattcctgcagctctgagtgtcccagaaggagaaaacttggttctcaactgcagtttcactgatagcgctatttacaacctccagtggtttaggcaggaccctgggaaaggtctcacatctctgttgcttattcagtcaagtcagagagagcaaacaagtggaagacttaatgcctcgctggataaatcatcaggacgtagtactttatacattgcagcttctcagcctggtgactcagccacctacctctgtgcctttataggccatggaggaagccaaggaaatctcatctttggaagaggaaccagccttattgttcatccgtatatccagaaccctgaccctgccgtgtaccagctgagagactctaaatccagtgacaagtctgtctgcctattcaccgattttgattctcaaacaaatgtgtcacaaagtaaggattctgatgtgtatatcacagacaaaactgtgctagacatgaggtctatggacttcaagagcaacagtgctgtggcctggagcaacaaatctgactttgcatgtgcaaacgccttcaacaacagcattattccagaagacaccttcttccccagcccagaaagttcctgtgatgtcaagctggtcgagaaaagctttgaaacagatacgaacctaaactttcaaaacctgtcagtgattgggttccgaatcctcctcctgaaagtggccgggtttaatctgctcatgacgctgcggctgtggtccagc

SEQ ID NO: 54 - DNA, 936 bp, Artificial Sequence
  T cell receptor beta TRBV19
atgagcatcggcctcctgtgctgtgcagccttgtctctcctgtgggcaggtccagtgaatgctggtgtcactcagaccccaaaattccaggtcctgaagacaggacagagcatgacactgcagtgtgcccaggatatgaaccatgaatacatgtcctggtatcgacaagacccaggcatggggctgaggctgattcattactcagttggtgctggtatcactgaccaaggagaagtccccaatggctacaatgtctccagatcaaccacagaggatttcccgctcaggctgctgtcggctgctccctcccagacatctgtgtacttctgtgccagtagtatgcagggggctatgagtgagcagttcttcggcccaggcacccggctgacagtgctcgaggacctgaaaaacgtgttcccacccgaggtcgctgtgtttgagccatcagaagcagagatctcccacacccaaaaggccacactggtatgcctggccacaggcttctaccccgaccacgtggagctgagctggtgggtgaatgggaaggaggtgcacagtggggtcagcacagacccgcagcccctcaaggagcagcccgccctcaatgactccagatactgcctgagcagccgcctgagggtctcggccaccttctggcagaacccccgcaaccacttccgctgtcaagtccagttctacgggctctcggagaatgacgagtggacccaggatagggccaaacccgtcacccagatcgtcagcgccgaggcctggggtagagcagactgtggcttcacctccgagtcttaccagcaaggggtcctgtctgccaccatcctctatgagatcttgctagggaaggccaccttgtatgccgtgctggtcagtgccctcgtgctgatggccatggtcaagagaaaggattccagaggctag

SEQ ID NO: 55 - protein, 270 aa, Artificial Sequence
  T cell receptor alpha TRAV23 DV6
METLLGLLILWLQLQWVSSKQEVTQIPAALSVPEGENLVLNCSFTDSAIYNLQWFRQDPGKGLTSLLLIQSSQREQTSGRLNASLDKSSGRSTLYIAASQPGDSATYLCAATGTYKYIFGRGTSLIVHPYIQNPDPAVYQLRDSKSSDKSVCLFTDFDSQTNVSQSKDSDVYITDKTVLDMRSMDFKSNSAVAWSNKSDFACANAFNNSIIPEDTFFPSPESSCDVKLVEKSFETDTNLNFQNLSVIGFRILLLKVAGFNLLMTLRLWSS

SEQ ID NO: 56 - protein, 315 aa, Artificial Sequence
  T cell receptor beta TRBV18
MSIGLLCCAALSLLWAGPVNAGVTQTPKFQVLKTGQSMTLQCAQDMNHEYMSWYRQDPGMGLRLIHYSVGAGITDQGEVPNGYNVSRSTTEDFPLRLLSAAPSQTSVYFCASSPEFARALDNQPQHFGPGTRLTVLEDLKNVFPPEVAVFEPSEAEISHTQKATLVCLATGFYPDHVELSWWVNGKEVHSGVSTDPQPLKEQPALNDSRYCLSSRLRVSATFWQNPRNHFRCQVQFYGLSENDEWTQDRAKPVTQIVSAEAWGRADCGFTSESYQQGVLSATILYEILLGKATLYAVLVSALVLMAMVKRKDSRG

SEQ ID NO: 57 - protein, 274 aa, Artificial Sequence
  T cell receptor alpha TRAV24
METLLGLLILWLQLQWVSSKQEVTQIPAALSVPEGENLVLNCSFTDSAIYNLQWFRQDPGKGLTSLLLIQSSQREQTSGRLNASLDKSSGRSTLYIAASQPGDSATYLCAFIGHGGSQGNLIFGRGTSLIVHPYIQNPDPAVYQLRDSKSSDKSVCLFTDFDSQTNVSQSKDSDVYITDKTVLDMRSMDFKSNSAVAWSNKSDFACANAFNNSIIPEDTFFPSPESSCDVKLVEKSFETDTNLNFQNLSVIGFRILLLKVAGFNLLMTLRLWSS

SEQ ID NO: 58 - protein, 311 aa, Artificial Sequence
  T cell receptor beta TRBV19
MSIGLLCCAALSLLWAGPVNAGVTQTPKFQVLKTGQSMTLQCAQDMNHEYMSWYRQDPGMGLRLIHYSVGAGITDQGEVPNGYNVSRSTTEDFPLRLLSAAPSQTSVYFCASSMQGAMSEQFFGPGTRLTVLEDLKNVFPPEVAVFEPSEAEISHTQKATLVCLATGFYPDHVELSWWVNGKEVHSGVSTDPQPLKEQPALNDSRYCLSSRLRVSATFWQNPRNHFRCQVQFYGLSENDEWTQDRAKPVTQIVSAEAWGRADCGFTSESYQQGVLSATILYEILLGKATLYAVLVSALVLMAMVKRKDSRG